European Patent Specification EP 3 992 287 B1, published October 9, 2024. Title: Antigen and Antibodies Prepared Based on PADI4 Serving as Tumor Maker, and Application Thereof. Applicant: Shandong Xinchuang Biotechnology Co., Ltd. The sequence listing filed with the application follows.

SEQUENCE LISTING (12 sequences)

SEQ ID NO: 1 - protein, 695 aa, Artificial synthesis
MGASWSHPQFEKGGGSGGGSGGSAWSHPQFEKMAQGTLIRVTPEQPTHAVCVLGTLTQLDICSSAPEDCTSFSINASPGVVVDIAHGPPAKKKSTGSSTWPLDPGVEVTLTMKVASGSTGDQKVQISYYGPKTPPVKALLYLTGVEISLCADITRTGKVKPTRAVKDQRTWTWGPCGQGAILLVNCDRDNLESSAMDCEDDEVLDSEDLQDMSLMTLSTKTPKDFFTNHTLVLHVARSEMDKVRVFQATRGKLSSKCSVVLGPKWPSHYLMVPGGKHNMDFYVEALAFPDTDFPGLITLTISLLDTSNLELPEAVVFQDSVVFRVAPWIMTPNTQPPQEVYACSIFENEDFLKSVTTLAMKAKCKLTICPEEENMDDQWMQDEMEIGYIQAPHKTLPVVFDSPRNRGLKEFPIKRVMGPDFGYVTRGPQTGGISGLDSFGNLEVSPPVTVRGKEYPLGRILFGDSCYPSNDSRQMHQALQDFLSAQQVQAPVKLYSDWLSVGHVDEFLSFVPAPDRKGFRLLLASPRSCYKLFQEQQNEGHGEALLFEGIKKKKQQKIKNILSNKTLREHNSFVERCIDWNRELLKRELGLAESDIIDIPQLFKLKEFSKAEAFFPNMVNMLVLGKHLGIPKPFGPVINGRCCLEEKVCSLLEPLGLQCTFINDFFTYHIRHGEVHCGTNVRRKPFSFKWWNMVP

SEQ ID NO: 2 - DNA, 2109 bp, Artificial synthesis
gaattcgccgccaccatgggcgcttcctggagccacccccagttcgagaagggtggtggcagcggtggcggcagcggaggttcagcttggtcccaccctcagttcgaaaagatggcccagggtactctgatccgtgtcacccccgagcagcctacccacgccgtctgcgtgctgggtaccctgactcagctggacatctgctccagcgctcctgaggactgcacttccttcagcatcaacgcttcccctggtgtcgtcgtggacatcgcccacggtcctcccgccaagaagaagtccaccggtagcagcacttggcctctggaccctggtgtggaggtcaccctgactatgaaggtggcttccggcagcaccggcgaccagaaggtccagatcagctactacggtcctaagaccccccccgtgaaggctctgctgtacctgactggcgtcgagatcagcctgtgcgctgacatcacccgtactggcaaggtgaagcctacccgtgctgtgaaggaccagcgcacttggacctggggcccttgcggtcagggtgctatcctgctggtcaactgcgaccgtgacaacctggagtcctccgctatggactgcgaagacgacgaagtgctggacagcgaggacctgcaggacatgtccctgatgactctgagcactaagactcccaaggacttcttcaccaaccacaccctggtcctgcacgtcgcccgcagcgagatggacaaggtgcgcgtcttccaggctacccgcggtaaactgtcctccaagtgcagcgtcgtgctgggccctaagtggccttcccactacctgatggtccccggtggtaaacacaacatggacttctacgtcgaggccctggccttccctgacactgacttccctggtctgatcactctgaccatctccctgctggacactagcaacctggaactgcccgaggccgtggtgttccaggacagcgtcgtgttccgtgtggctccctggatcatgacccccaacacccagccccctcaggaagtgtacgcttgcagcatcttcgaaaacgaggacttcctgaagagcgtcactaccctggctatgaaggccaagtgcaagctgaccatctgccctgaggaagagaacatggacgaccagtggatgcaggacgaaatggagatcggctacatccaggctcctcacaagactctgcccgtcgtgttcgacagcccccgtaaccgcggtctgaaggaatttcccatcaagcgcgtgatgggccctgacttcggttacgtgacccgtggtccccagactggcggtatctccggcctggacagcttcggcaacctggaggtctccccccctgtgactgtgcgcggcaaggagtaccccctgggtcgcatcctgttcggcgactcctgctacccttccaacgactcccgtcagatgcaccaggctctgcaggacttcctgagcgcccagcaggtgcaggctcctgtgaagctgtacagcgactggctgagcgtcggtcacgtcgacgagttcctgtccttcgtgcctgcccctgaccgcaagggcttccgcctgctgctggccagccccagatcctgctacaagctgttccaggagcagcagaacgaaggccacggtgaggctctgctgttcgaaggcatcaagaagaagaagcagcagaagatcaagaacatcctgagcaacaagactctgcgcgaacacaactccttcgtcgaacgttgcatcgactggaaccgtgaactgctgaagcgcgagctgggcctggccgagagcgacatcatcgacatccctcagctgttcaagctgaaggaattttctaaggccgaagcctttttccctaacatggtgaacatgctggtgctgggtaaacacctgggtatccctaagcccttcggtcccgtcatcaacggccgctgctgcctggaggagaaggtctgctccctgctggagcccctgggtctgcagtgcaccttcatcaacgacttcttcacttaccacatccgtcacggcgaagtgcactgcggtaccaacgtgcgccgcaagcctttctccttcaagtggtggaacatggtgccttaaaagctt

SEQ ID NO: 3 - protein, 469 aa, Artificial synthesis
MKHLWFFLLLVAAPRWVLSEVKLQESGPGILQPSQTLSLTCSFSGFSLSTSGMCVGWIRQPSGKGLEWLAHIWWDDDKRYNPALKSRLTISKDTSSNQVFLKIASVDTADTATYYCARYYRFDEGFDYWGQGTTLTVSSASTKGPSVFPLAPSSKSTSGGTAALGCLVKDYFPEPVTVSWNSGALTSGVHTFPAVLQSSGLYSLSSVVTVPSSSLGTQTYICNVNHKPSNTKVDKKVEPKSCDKTHTCPPCPAPELLGGPSVFLFPPKPKDTLMISRTPEVTCVVVDVSHEDPEVKFNWYVDGVEVHNAKTKPREEQYNSTYRVVSVLTVLHQDWLNGKEYKCKVSNKALPAPIEKTISKAKGQPREPQVYTLPPSREEMTKNQVSLTCLVKGFYPSDIAVEWESNGQPENNYKTTPPVLDSDGSFFLYSKLTVDKSRWQQGNVFSCSVMHEALHNHYTQKSLSLSPGK

SEQ ID NO: 4 - DNA, 1419 bp, Artificial synthesis
gccgccaccatgaagcacctgtggttctttctgctgctggtggccgctcctagatgggtgctgagcgaggtgaagctgcaggagtcaggacctgggatattgcagccctcccagaccctcagtctgacttgttctttctctgggttttcactgagcacttctggtatgtgtgtaggctggattcgtcagccttcagggaagggtctggagtggctggcacacatttggtgggatgatgacaagcgctataacccagcccttaagagccgactgacaatctccaaggatacctccagcaaccaggttttcctcaagatcgccagtgtggacactgcagatactgccacatactactgtgctcgatactataggttcgacgaagggtttgactactggggccaaggcaccactctcacagtctcctcagctagcaccaagggaccttctgtgttccctctggctccttcttctaagtccacttccggtggtacagcagctctgggttgtctggtgaaggattacttcccagaaccagtgactgtgtcctggaactccggagctctgacttctggagtgcatactttcccagcagtgctgcaatctagcggactgtactctctgtcttccgtggtgactgtgccttcttcttccctggggactcaaacttacatctgcaacgtgaaccacaagccctccaacaccaaggtggacaagaaggtggagccaaagagctgcgataagacccacacctgtccaccttgtccagctccagaactgctgggtgggccttctgtgtttctgttcccacctaagccaaaggataccctgatgatctctaggaccccagaagtgacctgtgtggtcgtcgatgtgtctcatgaagaccctgaagtgaagttcaactggtacgtggacggggtggaagtgcataacgcaaagaccaagcccagggaagagcaatacaactccacctacagggtggtctccgtcctgacagtcctgcatcaggattggctgaacggcaaggagtacaagtgcaaggtctccaataaagccctgcctgcccctatcgagaaaaccattagcaaagccaaaggccagcccagggagccccaggtctatacactgccccccagcagggaggagatgacaaaaaatcaggtcagcctgacatgcctggtcaaaggcttttatcccagcgacattgccgtcgagtgggagtccaatggccagcccgagaataattataaaacaacaccccccgtcctggacagcgacggcagcttttttctgtatagcaaactgacagtcgataaaagcaggtggcagcagggcaatgtcttttcctgcagcgtcatgcacgaggccctgcacaatcactatactcagaaaagcctgagcctgtcccccgggaaatga

SEQ ID NO: 5 - protein, 239 aa, Artificial synthesis
MVLQTQVFISLLLWISGAYGDIVITQDELSNPVTLGTSASISCRSSKSLLHSDGITYLYWYLQKPGQSPQLLIYQMSNLASGVPDRFSSSGSGTDFTLRISRVEAEDVGVYYCAQNLELPLTFGAGTKLELKRTVAAPSVFIFPPSDEQLKSGTASVVCLLNNFYPREAKVQWKVDNALQSGNSQESVTEQDSKDSTYSLSSTLTLSKADYEKHKVYACEVTHQGLSSPVTKSFNRGEC

SEQ ID NO: 6 - DNA, 729 bp, Artificial synthesis
gccgccaccatggtgctgcagacccaggtgttcatctctctgctgctgtggatctccggcgcctacggcgatatcgtgataacccaagatgaactctccaatccagtcactcttggaacatcagcttccatctcctgcaggtctagtaagagtctcctacatagtgatggcatcacttatttgtattggtatctgcagaagccaggccagtctcctcagctcctgatttatcagatgtccaaccttgcctcaggagtcccagacaggttcagtagcagtgggtcaggaactgatttcacactgagaatcagcagagtggaggctgaggatgtgggtgtttattactgtgctcaaaatctagaacttccgctcacgttcggtgctgggaccaagctggagctgaaacgtacggtggctgcaccttctgtgttcatcttccctccatctgatgagcagctgaagtctggaaccgcatctgtcgtctgtctgctgaacaacttttaccccagggaggctaaggtccaatggaaggtggacaacgccctgcagtctggtaatagccaggaaagcgtgaccgaacaggattccaaggactccacctactccctgtcctccacactgacactgagcaaagccgactatgaaaagcacaaagtgtatgcctgcgaggtcactcatcagggcctgtccagccccgtgactaaaagctttaataggggggagtgctga

SEQ ID NO: 7 - protein, 463 aa, Artificial synthesis
MKHLWFFLLLVAAPRWVLSEVKLQESGPSLVAPSQNLSITCTVSGFSLTSYAVHWFRQPPGKGLEWLGVIWAGGSTNCNSALMSRLSISKDNSKSQVFLKMNSLQTDDTAMYYCAREAGIPFDYWGQGTTLTVASTKGPSVFPLAPSSKSTSGGTAALGCLVKDYFPEPVTVSWNSGALTSGVHTFPAVLQSSGLYSLSSVVTVPSSSLGTQTYICNVNHKPSNTKVDKKVEPKSCDKTHTCPPCPAPELLGGPSVFLFPPKPKDTLMISRTPEVTCVVVDVSHEDPEVKFNWYVDGVEVHNAKTKPREEQYNSTYRVVSVLTVLHQDWLNGKEYKCKVSNKALPAPIEKTISKAKGQPREPQVYTLPPSREEMTKNQVSLTCLVKGFYPSDIAVEWESNGQPENNYKTTPPVLDSDGSFFLYSKLTVDKSRWQQGNVFSCSVMHEALHNHYTQKSLSLSPGK

SEQ ID NO: 8 - DNA, 1401 bp, Artificial synthesis
gccgccaccatgaagcacctgtggttctttctgctgctggtggccgctcctagatgggtgctgagcgaggtgaagctgcaggagtcaggacctagcctggtggctccatcccagaacctgagcatcacctgcacagtgtccggcttcagcctgacctcttacgctgtgcattggtttaggcagccacctggcaagggactggagtggctgggcgtgatctgggctggaggctccacaaactgcaattctgctctgatgtcccggctgtctatctccaaggacaacagcaagtctcaggtgttcctgaagatgaactccctgcagaccgacgatacagccatgtactattgtgcccgcgaggctggcatcccatttgattattggggccagggcaccacactgaccgtggctagcaccaagggaccttctgtgttccctctggctccttcttctaagtccacttccggtggtacagcagctctgggttgtctggtgaaggattacttcccagaaccagtgactgtgtcctggaactccggagctctgacttctggagtgcatactttcccagcagtgctgcaatctagcggactgtactctctgtcttccgtggtgactgtgccttcttcttccctggggactcaaacttacatctgcaacgtgaaccacaagccctccaacaccaaggtggacaagaaggtggagccaaagagctgcgataagacccacacctgtccaccttgtccagctccagaactgctgggtgggccttctgtgtttctgttcccacctaagccaaaggataccctgatgatctctaggaccccagaagtgacctgtgtggtcgtcgatgtgtctcatgaagaccctgaagtgaagttcaactggtacgtggacggggtggaagtgcataacgcaaagaccaagcccagggaagagcaatacaactccacctacagggtggtctccgtcctgacagtcctgcatcaggattggctgaacggcaaggagtacaagtgcaaggtctccaataaagccctgcctgcccctatcgagaaaaccattagcaaagccaaaggccagcccagggagccccaggtctatacactgccccccagcagggaggagatgacaaaaaatcaggtcagcctgacatgcctggtcaaaggcttttatcccagcgacattgccgtcgagtgggagtccaatggccagcccgagaataattataaaacaacaccccccgtcctggacagcgacggcagcttttttctgtatagcaaactgacagtcgataaaagcaggtggcagcagggcaatgtcttttcctgcagcgtcatgcacgaggccctgcacaatcactatactcagaaaagcctgagcctgtcccccgggaaatga

SEQ ID NO: 9 - protein, 466 aa, Artificial synthesis
MKHLWFFLLLVAAPRWVLSEVQLQESGPELEKPGASVKISCKASGYSFTGYNMNWVKQRNGKSLEWIGNIDPYNGGTNYNQKFKGKATLSVDKSSTTAYMQLKGLTSEDSAVYFCARETYYGDAMDYWGQGTSVTVASTKGPSVFPLAPSSKSTSGGTAALGCLVKDYFPEPVTVSWNSGALTSGVHTFPAVLQSSGLYSLSSVVTVPSSSLGTQTYICNVNHKPSNTKVDKKVEPKSCDKTHTCPPCPAPELLGGPSVFLFPPKPKDTLMISRTPEVTCVVVDVSHEDPEVKFNWYVDGVEVHNAKTKPREEQYNSTYRVVSVLTVLHQDWLNGKEYKCKVSNKALPAPIEKTISKAKGQPREPQVYTLPPSREEMTKNQVSLTCLVKGFYPSDIAVEWESNGQPENNYKTTPPVLDSDGSFFLYSKLTVDKSRWQQGNVFSCSVMHEALHNHYTQKSLSLSPGK

SEQ ID NO: 10 - DNA, 1410 bp, Artificial synthesis
gccgccaccatgaagcacctgtggttctttctgctgctggtggccgctcctagatgggtgctgagcgaggtgcagctgcaggagtcaggccctgagctggagaagcccggcgctagcgtgaagatcagctgcaaggcctccggctactccttcaccggctacaatatgaattgggtgaagcagagaaacggcaagagcctggagtggatcggcaacatcgatccttacaacggcggcacaaattacaatcagaagttcaagggcaaggccaccctgtccgtggataagagcagcacaaccgcctacatgcagctgaagggcctgacatccgaggactccgccgtgtacttttgcgccagggagacctactacggcgacgccatggattactggggccagggcaccagcgtgacagtggctagcaccaagggaccttctgtgttccctctggctccttcttctaagtccacttccggtggtacagcagctctgggttgtctggtgaaggattacttcccagaaccagtgactgtgtcctggaactccggagctctgacttctggagtgcatactttcccagcagtgctgcaatctagcggactgtactctctgtcttccgtggtgactgtgccttcttcttccctggggactcaaacttacatctgcaacgtgaaccacaagccctccaacaccaaggtggacaagaaggtggagccaaagagctgcgataagacccacacctgtccaccttgtccagctccagaactgctgggtgggccttctgtgtttctgttcccacctaagccaaaggataccctgatgatctctaggaccccagaagtgacctgtgtggtcgtcgatgtgtctcatgaagaccctgaagtgaagttcaactggtacgtggacggggtggaagtgcataacgcaaagaccaagcccagggaagagcaatacaactccacctacagggtggtctccgtcctgacagtcctgcatcaggattggctgaacggcaaggagtacaagtgcaaggtctccaataaagccctgcctgcccctatcgagaaaaccattagcaaagccaaaggccagcccagggagccccaggtctatacactgccccccagcagggaggagatgacaaaaaatcaggtcagcctgacatgcctggtcaaaggcttttatcccagcgacattgccgtcgagtgggagtccaatggccagcccgagaataattataaaacaacaccccccgtcctggacagcgacggcagcttttttctgtatagcaaactgacagtcgataaaagcaggtggcagcagggcaatgtcttttcctgcagcgtcatgcacgaggccctgcacaatcactatactcagaaaagcctgagcctgtcccccgggaaatga

SEQ ID NO: 11 - protein, 238 aa, Artificial synthesis
MVLQTQVFISLLLWISGAYGDIVLTQSPASLVVSLGQRATISCRASESVDSYGNSFMHWYQQKPGQPPKLLIYRASNLESGIPARFSGSGSRTDFTLTINPVEADDVATYYCQQTNEDPFTFGSGTKLEIKRTVAAPSVFIFPPSDEQLKSGTASVVCLLNNFYPREAKVQWKVDNALQSGNSQESVTEQDSKDSTYSLSSTLTLSKADYEKHKVYACEVTHQGLSSPVTKSFNRGEC

SEQ ID NO: 12 - DNA, 726 bp, Artificial synthesis
gccgccaccatggtgctgcagacccaggtgttcatctctctgctgctgtggatctccggcgcctacggcgacattgtgctgacccaatctccagcttctttggttgtgtctctagggcagagggccaccatatcctgcagagccagtgaaagtgttgatagttatggcaatagttttatgcactggtatcagcagaaaccaggacagccacccaaactcctcatctatcgtgcatccaacctagaatctgggatccctgccaggttcagtggcagtgggtctaggacagacttcaccctcaccattaatcctgtggaggctgatgatgttgcaacctattactgtcagcaaactaatgaggatccattcacgttcggctcggggacaaagttggaaataaaacgtacggtggctgcaccttctgtgttcatcttccctccatctgatgagcagctgaagtctggaaccgcatctgtcgtctgtctgctgaacaacttttaccccagggaggctaaggtccaatggaaggtggacaacgccctgcagtctggtaatagccaggaaagcgtgaccgaacaggattccaaggactccacctactccctgtcctccacactgacactgagcaaagccgactatgaaaagcacaaagtgtatgcctgcgaggtcactcatcagggcctgtccagccccgtgactaaaagctttaataggggggagtgctga